European Patent Application EP 4 796 634 A1, published August 26, 2026. Title: ANTISENSE OLIGONUCLEOTIDES (ASOS) FOR TREATMENT OF CARDIAC DISORDERS. Applicant: Hannover Medical School (MHH). Application EP. The sequence listing filed with the application follows.

SEQUENCE LISTING (59 sequences)

SEQ ID NO: 1 - DNA, 16 bp, synthetic construct
  misc_feature 4..13: note = DNA
  misc_feature order(1..3,14..16): note = RNA
  source 1..16: mol_type = other DNA
cgccgccatatctccc

SEQ ID NO: 2 - DNA, 16 bp, synthetic construct
  misc_feature 4..13: note = DNA
  misc_feature order(1..3,14..16): note = RNA
  source 1..16: mol_type = other DNA
cggacaaaactggttg

SEQ ID NO: 3 - DNA, 17 bp, synthetic construct
  misc_feature 4..14: note = DNA
  misc_feature order(1..3,15..17): note = RNA
  source 1..17: mol_type = other DNA
aagagtctcctccttaa

SEQ ID NO: 4 - DNA, 17 bp, synthetic construct
  misc_feature 4..14: note = DNA
  misc_feature order(1..3,15..17): note = RNA
  source 1..17: mol_type = other DNA
gattagccctgtgttca

SEQ ID NO: 5 - DNA, 17 bp, synthetic construct
  misc_feature 4..14: note = DNA
  misc_feature order(1..3,15..17): note = RNA
  source 1..17: mol_type = other DNA
cggcacaagagccaaag

SEQ ID NO: 6 - DNA, 17 bp, synthetic construct
  misc_feature 4..14: note = DNA
  misc_feature order(1..3,15..17): note = RNA
  source 1..17: mol_type = other DNA
tctcctccttaagcccc

SEQ ID NO: 7 - DNA, 17 bp, synthetic construct
  misc_feature 4..14: note = DNA
  misc_feature order(1..3,15..17): note = RNA
  source 1..17: mol_type = other DNA
gtctcctccttaagccc

SEQ ID NO: 8 - DNA, 16 bp, synthetic construct
  misc_feature 4..13: note = DNA
  misc_feature order(1..3,14..16): note = RNA
  misc_feature order(4,6..7,12): note = 5-methyl
  source 1..16: mol_type = other DNA
cgccgccatatctccc

SEQ ID NO: 9 - DNA, 16 bp, synthetic construct
  misc_feature 4..13: note = DNA
  misc_feature order(1..3,14..16): note = RNA
  misc_feature order(5,10): note = 5-methyl
  source 1..16: mol_type = other DNA
cggacaaaactggttg

SEQ ID NO: 10 - DNA, 17 bp, synthetic construct
  misc_feature 4..14: note = DNA
  misc_feature order(1..3,15..17): note = RNA
  misc_feature order(7,9..10,12..13): note = 5-methyl
  source 1..17: mol_type = other DNA
aagagtctcctccttaa

SEQ ID NO: 11 - DNA, 17 bp, synthetic construct
  misc_feature 4..14: note = DNA
  misc_feature order(1..3,15..17): note = RNA
  misc_feature 7..9: note = 5-methyl
  source 1..17: mol_type = other DNA
gattagccctgtgttca

SEQ ID NO: 12 - DNA, 17 bp, synthetic construct
  misc_feature 4..14: note = DNA
  misc_feature order(1..3,15..17): note = RNA
  misc_feature order(4,6,12..13): note = 5-methyl
  source 1..17: mol_type = other DNA
cggcacaagagccaaag

SEQ ID NO: 13 - DNA, 17 bp, synthetic construct
  misc_feature 4..14: note = DNA
  misc_feature order(1..3,15..17): note = RNA
  misc_feature order(4..5,7..8,14): note = 5-methyl
  source 1..17: mol_type = other DNA
tctcctccttaagcccc

SEQ ID NO: 14 - DNA, 17 bp, synthetic construct
  misc_feature 4..14: note = DNA
  misc_feature order(1..3,15..17): note = RNA
  misc_feature order(5..6,8..9): note = 5-methyl
  source 1..17: mol_type = other DNA
gtctcctccttaagccc

SEQ ID NO: 15 - DNA, 16 bp, synthetic construct
  misc_feature 4..13: note = DNA
  misc_feature order(1..3,14..16): note = RNA
  misc_feature order(1..3,14..16): note = LNA
  misc_feature order(4,6..7,12): note = 5-methyl
  source 1..16: mol_type = other DNA
cgccgccatatctccc

SEQ ID NO: 16 - DNA, 16 bp, synthetic construct
  misc_feature 4..13: note = DNA
  misc_feature order(1..3,14..16): note = RNA
  misc_feature order(1..3,14..16): note = LNA
  misc_feature order(5,10): note = 5-methyl
  source 1..16: mol_type = other DNA
cggacaaaactggttg

SEQ ID NO: 17 - DNA, 17 bp, synthetic construct
  misc_feature 4..14: note = DNA
  misc_feature order(1..3,15..17): note = RNA
  misc_feature order(1..3,15..17): note = LNA
  misc_feature order(7,9..10,12..13): note = 5-methyl
  source 1..17: mol_type = other DNA
aagagtctcctccttaa

SEQ ID NO: 18 - DNA, 17 bp, synthetic construct
  misc_feature 4..14: note = DNA
  misc_feature order(1..3,15..17): note = RNA
  misc_feature order(1..3,15..17): note = LNA
  misc_feature 7..9: note = 5-methyl
  source 1..17: mol_type = other DNA
gattagccctgtgttca

SEQ ID NO: 19 - DNA, 17 bp, synthetic construct
  misc_feature 4..14: note = DNA
  misc_feature order(1..3,15..17): note = RNA
  misc_feature order(1..3,15..17): note = LNA
  misc_feature order(4,6,12..13): note = 5-methyl
  source 1..17: mol_type = other DNA
cggcacaagagccaaag

SEQ ID NO: 20 - DNA, 17 bp, synthetic construct
  misc_feature 4..14: note = DNA
  misc_feature order(1..3,15..17): note = RNA
  misc_feature order(1..3,15..17): note = LNA
  misc_feature order(4..5,7..8,14): note = 5-methyl
  source 1..17: mol_type = other DNA
tctcctccttaagcccc

SEQ ID NO: 21 - DNA, 17 bp, synthetic construct
  misc_feature 4..14: note = DNA
  misc_feature order(1..3,15..17): note = RNA
  misc_feature order(1..3,15..17): note = LNA
  misc_feature order(5..6,8..9): note = 5-methyl
  source 1..17: mol_type = other DNA
gtctcctccttaagccc

SEQ ID NO: 22 - DNA, 16 bp, synthetic construct
  misc_feature 4..13: note = DNA
  misc_feature order(1..3,14..16): note = RNA
  misc_feature order(1..3,14..16): note = LNA
  misc_feature order(4,6..7,12): note = 5-methyl
  modified_base 1..16: mod_base = OTHER; note = phosphorothioate
  source 1..16: mol_type = other DNA
cgccgccatatctccc

SEQ ID NO: 23 - DNA, 16 bp, synthetic construct
  misc_feature 4..13: note = DNA
  misc_feature order(1..3,14..16): note = RNA
  misc_feature order(1..3,14..16): note = LNA
  misc_feature order(5,10): note = 5-methyl
  modified_base 1..16: mod_base = OTHER; note = phosphorothioate
  source 1..16: mol_type = other DNA
cggacaaaactggttg

SEQ ID NO: 24 - DNA, 17 bp, synthetic construct
  misc_feature 4..14: note = DNA
  misc_feature order(1..3,15..17): note = RNA
  misc_feature order(1..3,15..17): note = LNA
  misc_feature order(7,9..10,12..13): note = 5-methyl
  modified_base 1..17: mod_base = OTHER; note = phosphorothioate
  source 1..17: mol_type = other DNA
aagagtctcctccttaa

SEQ ID NO: 25 - DNA, 17 bp, synthetic construct
  misc_feature 4..14: note = DNA
  misc_feature order(1..3,15..17): note = RNA
  misc_feature order(1..3,15..17): note = LNA
  misc_feature 7..9: note = 5-methyl
  source 1..17: mol_type = other DNA
  modified_base 1..17: mod_base = OTHER; note = phosphorothioate
gattagccctgtgttca

SEQ ID NO: 26 - DNA, 17 bp, synthetic construct
  misc_feature 4..14: note = DNA
  misc_feature order(1..3,15..17): note = RNA
  misc_feature order(1..3,15..17): note = LNA
  misc_feature order(4,6,12..13): note = 5-methyl
  source 1..17: mol_type = other DNA
  modified_base 1..17: mod_base = OTHER; note = phosphorothioate
cggcacaagagccaaag

SEQ ID NO: 27 - DNA, 17 bp, synthetic construct
  misc_feature 4..14: note = DNA
  misc_feature order(1..3,15..17): note = RNA
  misc_feature order(1..3,15..17): note = LNA
  misc_feature order(4..5,7..8,14): note = 5-methyl
  source 1..17: mol_type = other DNA
  modified_base 1..17: mod_base = OTHER; note = phosphorothioate
tctcctccttaagcccc

SEQ ID NO: 28 - DNA, 17 bp, synthetic construct
  misc_feature 4..14: note = DNA
  misc_feature order(1..3,15..17): note = RNA
  misc_feature order(1..3,15..17): note = LNA
  misc_feature order(5..6,8..9): note = 5-methyl
  source 1..17: mol_type = other DNA
  modified_base 1..17: mod_base = OTHER; note = phosphorothioate
gtctcctccttaagccc

SEQ ID NO: 29 - RNA, 19 nt, synthetic construct
  source 1..19: mol_type = other RNA
cagtcaacgggggacataa

SEQ ID NO: 30 - RNA, 20 nt, synthetic construct
  source 1..20: mol_type = other RNA
gctgtactgcttgaccaagg

SEQ ID NO: 31 - RNA, 20 nt, synthetic construct
  source 1..20: mol_type = other RNA
atgccttacctggagctctc

SEQ ID NO: 32 - RNA, 20 nt, synthetic construct
  source 1..20: mol_type = other RNA
gttgcttgtccctcgatgtc

SEQ ID NO: 33 - RNA, 20 nt, synthetic construct
  source 1..20: mol_type = other RNA
acaacttctttccccgcaag

SEQ ID NO: 34 - RNA, 21 nt, synthetic construct
  source 1..21: mol_type = other RNA
gctccatacttttaaggcccg

SEQ ID NO: 35 - RNA, 19 nt, synthetic construct
  source 1..19: mol_type = other RNA
agtttccgtgcctggcccc

SEQ ID NO: 36 - RNA, 20 nt, synthetic construct
  source 1..20: mol_type = other RNA
acctcggggacccatctggc

SEQ ID NO: 37 - RNA, 20 nt, synthetic construct
  source 1..20: mol_type = other RNA
acacacgagacgctgaagta

SEQ ID NO: 38 - RNA, 20 nt, synthetic construct
  source 1..20: mol_type = other RNA
tccactcaggcatcgacatt

SEQ ID NO: 39 - RNA, 20 nt, synthetic construct
  source 1..20: mol_type = other RNA
ctctccgcaagagacttcca

SEQ ID NO: 40 - RNA, 20 nt, synthetic construct
  source 1..20: mol_type = other RNA
agtctcctctccggacttgt

SEQ ID NO: 41 - RNA, 20 nt, synthetic construct
  source 1..20: mol_type = other RNA
ccatcacatcgtagccctct

SEQ ID NO: 42 - RNA, 20 nt, synthetic construct
  source 1..20: mol_type = other RNA
tatatcgcccgttgactggt

SEQ ID NO: 43 - RNA, 20 nt, synthetic construct
  source 1..20: mol_type = other RNA
ggaggagcgttagcatcttg

SEQ ID NO: 44 - RNA, 20 nt, synthetic construct
  source 1..20: mol_type = other RNA
gacagtgggacagcctgttt

SEQ ID NO: 45 - RNA, 22 nt, synthetic construct
  source 1..22: mol_type = other RNA
ctgcttctggtgatggctactg

SEQ ID NO: 46 - RNA, 20 nt, synthetic construct
  source 1..20: mol_type = other RNA
ggcatcacctttggcatctt

SEQ ID NO: 47 - RNA, 21 nt, synthetic construct
  source 1..21: mol_type = other RNA
ccactcacagactctcacaac

SEQ ID NO: 48 - RNA, 21 nt, synthetic construct
  source 1..21: mol_type = other RNA
ctgcggtacaatcccagaact

SEQ ID NO: 49 - RNA, 20 nt, synthetic construct
  source 1..20: mol_type = other RNA
gaagaactgcggatggaagc

SEQ ID NO: 50 - RNA, 20 nt, synthetic construct
  source 1..20: mol_type = other RNA
cacgtaggcatccaggtgat

SEQ ID NO: 51 - RNA, 24 nt, synthetic construct
  source 1..24: mol_type = other RNA
tgacatcaagggcatttcaggagc

SEQ ID NO: 52 - RNA, 24 nt, synthetic construct
  source 1..24: mol_type = other RNA
gtccgccaaatgaaccggtccttg

SEQ ID NO: 53 - RNA, 20 nt, synthetic construct
  source 1..20: mol_type = other RNA
acgaagacatcccaccaatc

SEQ ID NO: 54 - RNA, 20 nt, synthetic construct
  source 1..20: mol_type = other RNA
cttggtcggtgggtgactct

SEQ ID NO: 55 - RNA, 21 nt, synthetic construct
  source 1..21: mol_type = other RNA
gaggatggttgcacgaaacac

SEQ ID NO: 56 - RNA, 20 nt, synthetic construct
  source 1..20: mol_type = other RNA
ggtagtctcacagccttgcg

SEQ ID NO: 57 - RNA, 28 nt, synthetic construct
  source 1..28: mol_type = other RNA
  misc_feature 28: note = biotinylated
ttaggtaagagggacagctggctggaaa

SEQ ID NO: 58 - RNA, 32 nt, synthetic construct
  source 1..32: mol_type = other RNA
  misc_feature 1: note = biotinylated
aaagacatcataagggtgatgacagagtcagt

SEQ ID NO: 59 - RNA, 15 nt, synthetic construct
  source 1..15: mol_type = other RNA
  modified_base 1..15: mod_base = OTHER; note = phosphorothioate
aacacgtctatacgc